European Patent Application EP 4 617 366 A1, published September 17, 2025. Title: Antibody for coatomer protein complex subunit beta 2. Applicant: ISM Co., Ltd. The sequence listing filed with the application follows.

SEQUENCE LISTING (24 sequences)

SEQ ID NO: 1 - protein, 8 aa, unidentified
  REGION 1..8: note = A2-7C6 Heavy chain CDR1
EFTFSRNG

SEQ ID NO: 2 - protein, 8 aa, unidentified
  REGION 1..8: note = A2-7C6 Heavy chain CDR2
ISSGGVST

SEQ ID NO: 3 - protein, 12 aa, unidentified
  REGION 1..12: note = A2-7C6 Heavy chain CDR3
CARHEGSRFAYW

SEQ ID NO: 4 - protein, 6 aa, unidentified
  REGION 1..6: note = A2-7C6 Light chain CDR1
QDINSY

SEQ ID NO: 5 - skipped

SEQ ID NO: 6 - protein, 11 aa, unidentified
  REGION 1..11: note = A2-7C6 Light chain CDR3
CLQYDEFPLTF

SEQ ID NO: 7 - protein, 8 aa, unidentified
  REGION 1..8: note = A2-7D11 Heavy chain CDR1
GFTFNNSA

SEQ ID NO: 8 - protein, 7 aa, unidentified
  REGION 1..7: note = A2-7D11 Heavy chain CDR2
ISNGGVT

SEQ ID NO: 9 - protein, 13 aa, unidentified
  REGION 1..13: note = A2-7D11 Heavy chain CDR3
CARGHYPYFFDYW

SEQ ID NO: 10 - protein, 6 aa, unidentified
  REGION 1..6: note = A2-7D11 Light chain CDR1
QDINNY

SEQ ID NO: 11 - skipped

SEQ ID NO: 12 - protein, 11 aa, unidentified
  REGION 1..11: note = A2-7D11 Light chain CDR3
CLQYDEFPLTF

SEQ ID NO: 13 - protein, 8 aa, unidentified
  REGION 1..8: note = A3-8C9 Heavy chain CDR1
GYTFTNYG

SEQ ID NO: 14 - protein, 8 aa, unidentified
INTYSGVA

SEQ ID NO: 15 - protein, 10 aa, unidentified
  REGION 1..10: note = A3-8C9 Heavy chain CDR3
CARADLFAYW

SEQ ID NO: 16 - protein, 11 aa, unidentified
  REGION 1..11: note = A3-8C9 Light chain CDR1
QSLVHSNGNTY

SEQ ID NO: 17 - skipped

SEQ ID NO: 18 - protein, 11 aa, unidentified
  REGION 1..11: note = A3-8C9 Light chain CDR3
CSQSTHVPRTF

SEQ ID NO: 19 - protein, 145 aa, unidentified
  REGION 1..145: note = A2-7C6 Heavy chain
MSTEHGPLTMNFGLSLIFLVLILKGVQCEVQLVESGGGLVKPGGSLKLSCAASEFTFSRNGMSWVRQTPAKRLEWVATISSGGVSTYYPDTVKGRFTISRDNAKNTLYLQMSSLRSEDTAMYYCARHEGSRFAYWGQGTLVTVSA

SEQ ID NO: 20 - protein, 143 aa, unidentified
  REGION 1..143: note = A2-7C6 Light chain
MQLESSSGVLPGLSMDMRTPAQFLGILLLWFPGIKCDIKMTQSPSSMYTSLGERVTITCKASQDINSYLSWFQQKPGNSPKTLIYLVNRLVDGVPSRFSGSGSGQDYSLTIGSLEFEDVGIYYCLQYDEFPLTFGAGTKLELK

SEQ ID NO: 21 - protein, 145 aa, unidentified
  REGION 1..145: note = A2-7D11 Heavy chain
MSTEHRHLTMNFGFSLIFLVLVLKGVQCEVKLVESGGGLVKPGGSLKLSCVASGFTFNNSAMSWVRQTPEKRLEWVSSISNGGVTFYPDNVKGRFTISRDDARDILYLQMSSLKSEDTAMYYCARGHYPYFFDYWGQGTTLTVSS

SEQ ID NO: 22 - protein, 129 aa, unidentified
  REGION 1..129: note = A2-7D11 Light chain
MDMRTPAQFLGILLLWFPGIKCDIKMTQSPSSMYASLGERVTITCKASQDINNYLSWFQQKPGKSPKTLIYRANRLVDGVPSRFSGSGSGRDYSLTISSLEYEDIGIYYCLQYDEFPLTFGAGTKLELK

SEQ ID NO: 23 - protein, 134 aa, unidentified
  REGION 1..134: note = A3-8C9 Heavy chain
MDWVWNLLFLMAAAQSIQAQIQLVQSGPELKKPGETVKISCKASGYTFTNYGMNWVKQAPGKGLKWMAWINTYSGVATHADDFKGRFDFSLETSASTAYLQINNLKNEDTATYFCARADLFAYWGQGTLVTVSA

SEQ ID NO: 24 - protein, 131 aa, unidentified
  REGION 1..131: note = A3-8C9 Light chain
MKLPVRLLVLMFWIPASSSDVVMTQTPLSLPVSLGDQASISCRSSQSLVHSNGNTYLHWYLQKPGQSPKLLIYKVSNRFSGVPDRFSGSGSGTDFTLKISRVEAEDLGVYFCSQSTHVPRTFGGGTKLEIK